European Patent Specification EP 3 936 142 B1, published January 17, 2024. Title: Therapeutic use of Trigonal glucagon/GLP-1/GIP receptor agonist or a conjugate thereof for liver disease. Applicant: HANMI PHARM. CO., LTD. The sequence listing filed with the application follows.

SEQUENCE LISTING (139 sequences)

SEQ ID NO: 1 - protein, 30 aa, Artificial Sequence
  Trigonal agonist
  MISC_FEATURE (2): Xaa is aminoisobutyric acid (Aib)
HXQGTFTSDVSSYLDGQAAKEFIAWLVKGC

SEQ ID NO: 2 - protein, 30 aa, Artificial Sequence
  Trigonal agonist
  MISC_FEATURE (2): Xaa is aminoisobutyric acid (Aib)
HXQGTFTSDVSSYLDGQAQKEFIAWLVKGC

SEQ ID NO: 3 - protein, 41 aa, Artificial Sequence
  Trigonal agonist
  MISC_FEATURE (2): Xaa is aminoisobutyric acid (Aib)
HXQGTFTSDVSSYLLGQAAKQFIAWLVKGGGPSSGAPPPSC

SEQ ID NO: 4 - protein, 30 aa, Artificial Sequence
  Trigonal agonist
  MISC_FEATURE (2): Xaa is aminoisobutyric acid (Aib)
HXQGTFTSDVSSYLLGQQQKEFIAWLVKGC

SEQ ID NO: 5 - protein, 41 aa, Artificial Sequence
  Trigonal agonist
  MISC_FEATURE (2): Xaa is aminoisobutyric acid (Aib)
HXQGTFTSDVSSYLLGQQQKEFIAWLVKGGGPSSGAPPPSC

SEQ ID NO: 6 - protein, 30 aa, Artificial Sequence
  Trigonal agonist
  MISC_FEATURE (2): Xaa is aminoisobutyric acid (Aib)
HXQGTFTSDVSSYLDGQAAKEFVAWLLKGC

SEQ ID NO: 7 - protein, 30 aa, Artificial Sequence
  Trigonal agonist
  MISC_FEATURE (2): Xaa is aminoisobutyric acid (Aib)
HXQGTFTSDVSKYLDGQAAKEFVAWLLKGC

SEQ ID NO: 8 - protein, 30 aa, Artificial Sequence
  Trigonal agonist
  MISC_FEATURE (2): Xaa is aminoisobutyric acid (Aib)
HXQGTFTSDVSKYLDGQAAQEFVAWLLKGC

SEQ ID NO: 9 - protein, 30 aa, Artificial Sequence
  Trigonal agonist
  MISC_FEATURE (2): Xaa is aminoisobutyric acid (Aib)
HXQGTFTSDVSKYLDGQAAQEFVAWLLAGC

SEQ ID NO: 10 - protein, 41 aa, Artificial Sequence
  Trigonal agonist
  MISC_FEATURE (2): Xaa is aminoisobutyric acid (Aib)
HXQGTFTSDVSKYLDGQAAQEFVAWLLAGGGPSSGAPPPSC

SEQ ID NO: 11 - protein, 41 aa, Artificial Sequence
  Trigonal agonist
  MISC_FEATURE (1): Xaa is 4-imidazoacetyl (CA)
XGEGTFTSDLSKYLDSRRQQLFVQWLKAGGPSSGAPPPSHG

SEQ ID NO: 12 - protein, 41 aa, Artificial Sequence
  Trigonal agonist
  MISC_FEATURE (1): Xaa is 4-imidazoacetyl (CA)
XGEGTFISDLSKYMDEQAVQLFVEWLMAGGPSSGAPPPSHG

SEQ ID NO: 13 - protein, 41 aa, Artificial Sequence
  Trigonal agonist
  MISC_FEATURE (1): Xaa is 4-imidazoacetyl (CA)
XGEGTFISDYSIQLDEIAVQDFVEWLLAQKPSSGAPPPSHG

SEQ ID NO: 14 - protein, 41 aa, Artificial Sequence
  Trigonal agonist
  MISC_FEATURE (1): Xaa is 4-imidazoacetyl (CA)
XGQGTFTSDYSIQLDEIAVRDFVEWLKNGGPSSGAPPPSHG

SEQ ID NO: 15 - protein, 41 aa, Artificial Sequence
  Trigonal agonist
  MISC_FEATURE (1): Xaa is 4-imidazoacetyl (CA)
XGQGTFTSDLSKQMDEEAVRLFIEWLKNGGPSSGAPPPSHG

SEQ ID NO: 16 - protein, 41 aa, Artificial Sequence
  Trigonal agonist
  MISC_FEATURE (1): Xaa is 4-imidazoacetyl (CA)
XGQGTFTSDLSKQMDSEAQQLFIEWLKNGGPSSGAPPPSHG

SEQ ID NO: 17 - protein, 41 aa, Artificial Sequence
  Trigonal agonist
  MISC_FEATURE (1): Xaa is 4-imidazoacetyl (CA)
XGQGTFTSDLSKQMDEERAREFIEWLLAQKPSSGAPPPSHG

SEQ ID NO: 18 - protein, 41 aa, Artificial Sequence
  Trigonal agonist
  MISC_FEATURE (1): Xaa is 4-imidazoacetyl (CA)
XGQGTFTSDLSKQMDSERAREFIEWLKNTGPSSGAPPPSHG

SEQ ID NO: 19 - protein, 41 aa, Artificial Sequence
  Trigonal agonist
  MISC_FEATURE (1): Xaa is 4-imidazoacetyl (CA)
XGQGTFTSDLSIQYDSEHQRDFIEWLKDTGPSSGAPPPSHG

SEQ ID NO: 20 - protein, 41 aa, Artificial Sequence
  Trigonal agonist
  MISC_FEATURE (1): Xaa is 4-imidazoacetyl (CA)
XGQGTFTSDLSIQYEEEAQQDFVEWLKDTGPSSGAPPPSHG

SEQ ID NO: 21 - protein, 39 aa, Artificial Sequence
  Trigonal agonist
  MISC_FEATURE (2): Xaa is aminoisobutyric acid (Aib)
  MISC_FEATURE (16)..(20): amino acids at positions 16 and 20 form a ring
YXQGTFTSDYSKYLDECRAKEFVQWLLDHHPSSGQPPPS

SEQ ID NO: 22 - protein, 39 aa, Artificial Sequence
  Trigonal agonist
  MISC_FEATURE (2): Xaa is aminoisobutyric acid (Aib)
  MISC_FEATURE (16)..(20): amino acids at positions 16 and 20 form a ring
YXQGTFTSDYSKCLDEKRAKEFVQWLLDHHPSSGQPPPS

SEQ ID NO: 23 - protein, 41 aa, Artificial Sequence
  Trigonal agonist
  MISC_FEATURE (2): Xaa is aminoisobutyric acid (Aib)
  MISC_FEATURE (16)..(20): amino acids at positions 16 and 20 form a ring
YXQGTFTSDYSKYLDECRAKEFVQWLLAQKGKKNDWKHNIT

SEQ ID NO: 24 - protein, 39 aa, Artificial Sequence
  Trigonal agonist
  MISC_FEATURE (2): Xaa is aminoisobutyric acid (Aib)
  MISC_FEATURE (16)..(20): amino acids at positions 16 and 20 form a ring
YXQGTFTSDYSKYLDECRAKEFVQWLKNGGPSSGAPPPS

SEQ ID NO: 25 - protein, 39 aa, Artificial Sequence
  Trigonal agonist
  MISC_FEATURE (2): Xaa is aminoisobutyric acid (Aib)
HXQGTFTSDCSKYLDERAAQDFVQWLLDGGPSSGAPPPS

SEQ ID NO: 26 - protein, 39 aa, Artificial Sequence
  Trigonal agonist
  MISC_FEATURE (2): Xaa is aminoisobutyric acid (Aib)
HXQGTFTSDCSKYLDSRAAQDFVQWLLDGGPSSGAPPPS

SEQ ID NO: 27 - protein, 40 aa, Artificial Sequence
  Trigonal agonist
  MISC_FEATURE (2): Xaa is aminoisobutyric acid (Aib)
HXQGTFTSDYSKYLDERACQDFVQWLLDQGGPSSGAPPPS

SEQ ID NO: 28 - protein, 41 aa, Artificial Sequence
  Trigonal agonist
  MISC_FEATURE (2): Xaa is aminoisobutyric acid (Aib)
HXQGTFTSDYSKYLDEKRAQEFVCWLLAQKGKKNDWKHNIT

SEQ ID NO: 29 - protein, 30 aa, Artificial Sequence
  Trigonal agonist
  MISC_FEATURE (2): Xaa is aminoisobutyric acid (Aib)
  MISC_FEATURE (16)..(20): amino acids at positions 16 and 20 form a ring
HXQGTFTSDYSKYLDEKAAKEFVQWLLNTC

SEQ ID NO: 30 - protein, 30 aa, Artificial Sequence
  Trigonal agonist
  MISC_FEATURE (2): Xaa is aminoisobutyric acid (Aib)
  MISC_FEATURE (16)..(20): amino acids at positions 16 and 20 form a ring
HXQGTFTSDYSKYLDEKAQKEFVQWLLDTC

SEQ ID NO: 31 - protein, 29 aa, Artificial Sequence
  Trigonal agonist
  MISC_FEATURE (2): Xaa is aminoisobutyric acid (Aib)
  MISC_FEATURE (16)..(20): amino acids at positions 16 and 20 form a ring
HXQGTFTSDYSKYLDEKACKEFVQWLLAQ

SEQ ID NO: 32 - protein, 39 aa, Artificial Sequence
  Trigonal agonist
  MISC_FEATURE (2): Xaa is aminoisobutyric acid (Aib)
  MISC_FEATURE (16)..(20): amino acids at positions 16 and 20 form a ring
HXQGTFTSDYSKYLDEKACKDFVQWLLDGGPSSGAPPPS

SEQ ID NO: 33 - protein, 31 aa, Artificial Sequence
  Trigonal agonist
  MISC_FEATURE (2): Xaa is aminoisobutyric acid (Aib)
  MISC_FEATURE (16)..(20): amino acids at positions 16 and 20 form a ring
HXQGTFTSDYSIAMDEIHQKDFVNWLLAQKC

SEQ ID NO: 34 - protein, 31 aa, Artificial Sequence
  Trigonal agonist
  MISC_FEATURE (2): Xaa is aminoisobutyric acid (Aib)
  MISC_FEATURE (16)..(20): amino acids at positions 16 and 20 form a ring
HXQGTFTSDYSKYLDEKRQKEFVNWLLAQKC

SEQ ID NO: 35 - protein, 31 aa, Artificial Sequence
  Trigonal agonist
  MISC_FEATURE (2): Xaa is aminoisobutyric acid (Aib)
  MISC_FEATURE (16)..(20): amino acids at positions 16 and 20 form a ring
HXQGTFTSDYSIAMDEIHQKDFVNWLLNTKC

SEQ ID NO: 36 - protein, 40 aa, Artificial Sequence
  Trigonal agonist
  MISC_FEATURE (2): Xaa is aminoisobutyric acid (Aib)
  MISC_FEATURE (16)..(20): amino acids at positions 16 and 20 form a ring
HXQGTFTSDYSKYLCEKRQKEFVQWLLNGGPSSGAPPPSG

SEQ ID NO: 37 - protein, 40 aa, Artificial Sequence
  Trigonal agonist
  MISC_FEATURE (2): Xaa is aminoisobutyric acid (Aib)
  MISC_FEATURE (16)..(20): amino acids at positions 16 and 20 form a ring
HXQGTFTSDYSKYLDECRQKEFVQWLLNGGPSSGAPPPSG

SEQ ID NO: 38 - protein, 40 aa, Artificial Sequence
  Trigonal agonist
  MISC_FEATURE (1): Xaa is 4-imidazoacetyl (CA)
  MISC_FEATURE (2): Xaa is aminoisobutyric acid (Aib)
XXQGTFTSDKSSYLDERAAQDFVQWLLDGGPSSGAPPPSS

SEQ ID NO: 39 - protein, 40 aa, Artificial Sequence
  Trigonal agonist
  MISC_FEATURE (2): Xaa is aminoisobutyric acid (Aib)
HXQGTFTSDYSKYLDGQHAQCFVAWLLAGGGPSSGAPPPS

SEQ ID NO: 40 - protein, 39 aa, Artificial Sequence
  Trigonal agonist
  MISC_FEATURE (2): Xaa is aminoisobutyric acid (Aib)
HXQGTFTSDKSKYLDERACQDFVQWLLDGGPSSGAPPPS

SEQ ID NO: 41 - protein, 39 aa, Artificial Sequence
  Trigonal agonist
  MISC_FEATURE (2): Xaa is aminoisobutyric acid (Aib)
HXQGTFTSDKSKYLDECAAQDFVQWLLDGGPSSGAPPPS

SEQ ID NO: 42 - protein, 40 aa, Artificial Sequence
  Trigonal agonist
  MISC_FEATURE (2): Xaa is aminoisobutyric acid (Aib)
  MISC_FEATURE (16)..(20): amino acids at positions 16 and 20 form a ring
YXQGTFTSDYSKYLDEKRAKEFVQWLLDHHPSSGQPPPSC

SEQ ID NO: 43 - protein, 39 aa, Artificial Sequence
  Trigonal agonist
  MISC_FEATURE (2): Xaa is aminoisobutyric acid (Aib)
  MISC_FEATURE (16)..(20): amino acids at positions 16 and 20 form a ring
YXQGTFTSDYSKYLDEKRAKEFVQWLLDHHCSSGQPPPS

SEQ ID NO: 44 - protein, 39 aa, Artificial Sequence
  Trigonal agonist
HGQGTFTSDCSKQLDGQAAQEFVAWLLAGGPSSGAPPPS

SEQ ID NO: 45 - protein, 39 aa, Artificial Sequence
  Trigonal agonist
HGQGTFTSDCSKYMDGQAAQDFVAWLLAGGPSSGAPPPS

SEQ ID NO: 46 - protein, 39 aa, Artificial Sequence
  Trigonal agonist
HGQGTFTSDCSKYLDEQHAQEFVAWLLAGGPSSGAPPPS

SEQ ID NO: 47 - protein, 39 aa, Artificial Sequence
  Trigonal agonist
HGQGTFTSDCSKYLDGQRAQEFVAWLLAGGPSSGAPPPS

SEQ ID NO: 48 - protein, 39 aa, Artificial Sequence
  Trigonal agonist
HGQGTFTSDCSKYLDGQRAQDFVNWLLAGGPSSGAPPPS

SEQ ID NO: 49 - protein, 30 aa, Artificial Sequence
  Trigonal agonist
  MISC_FEATURE (1): Xaa is 4-imidazoacetyl (CA)
  MISC_FEATURE (2): Xaa is aminoisobutyric acid (Aib)
  MISC_FEATURE (16)..(20): amino acids at positions 16 and 20 form a ring
XXQGTFTSDYSICMDEIHQKDFVNWLLNTK

SEQ ID NO: 50 - protein, 40 aa, Artificial Sequence
  Trigonal agonist
  MISC_FEATURE (2): Xaa is aminoisobutyric acid (Aib)
  MISC_FEATURE (16)..(20): amino acids at positions 16 and 20 form a ring
HXQGTFTSDYSKYLDEKRAKEFVQWLLDHHPSSGQPPPSC

SEQ ID NO: 51 - protein, 30 aa, Artificial Sequence
  Trigonal agonist
  MISC_FEATURE (2): Xaa is aminoisobutyric acid (Aib)
  MISC_FEATURE (16)..(20): amino acids at positions 16 and 20 form a ring
HXQGTFTSDYSKYLDEKRQKEFVQWLLNTC

SEQ ID NO: 52 - protein, 30 aa, Artificial Sequence
  Trigonal agonist
  MISC_FEATURE (2): Xaa is aminoisobutyric acid (Aib)
  MISC_FEATURE (16)..(20): amino acids at positions 16 and 20 form a ring
HXQGTFTSDYSKYLDEKRQKEFVQWLLDTC

SEQ ID NO: 53 - protein, 30 aa, Artificial Sequence
  Trigonal agonist
  MISC_FEATURE (2): Xaa is aminoisobutyric acid (Aib)
  MISC_FEATURE (16)..(20): amino acids at positions 16 and 20 form a ring
HXEGTFTSDYSIAMDEIHQKDFVNWLLAQC

SEQ ID NO: 54 - protein, 30 aa, Artificial Sequence
  Trigonal agonist
  MISC_FEATURE (2): Xaa is aminoisobutyric acid (Aib)
  MISC_FEATURE (16)..(20): amino acids at positions 16 and 20 form a ring
HXEGTFTSDYSIAMDEIHQKDFVDWLLAEC

SEQ ID NO: 55 - protein, 30 aa, Artificial Sequence
  Trigonal agonist
  MISC_FEATURE (2): Xaa is aminoisobutyric acid (Aib)
  MISC_FEATURE (16)..(20): amino acids at positions 16 and 20 form a ring
HXQGTFTSDYSIAMDEIHQKDFVNWLLAQC

SEQ ID NO: 56 - protein, 30 aa, Artificial Sequence
  Trigonal agonist
  MISC_FEATURE (2): Xaa is aminoisobutyric acid (Aib)
  MISC_FEATURE (16)..(20): amino acids at positions 16 and 20 form a ring
HXQGTFTSDYSKYLDEKRQKEFVNWLLAQC

SEQ ID NO: 57 - protein, 30 aa, Artificial Sequence
  Trigonal agonist
  MISC_FEATURE (2): Xaa is aminoisobutyric acid (Aib)
  MISC_FEATURE (16)..(20): amino acids at positions 16 and 20 form a ring
HXQGTFTSDYSIAMDEIHQKDFVNWLLNTC

SEQ ID NO: 58 - protein, 31 aa, Artificial Sequence
  Trigonal agonist
  MISC_FEATURE (2): Xaa is aminoisobutyric acid (Aib)
  MISC_FEATURE (16)..(20): amino acids at positions 16 and 20 form a ring
HXQGTFTSDYSKYLDEKRQKEFVQWLLNTKC

SEQ ID NO: 59 - protein, 30 aa, Artificial Sequence
  Trigonal agonist
  MISC_FEATURE (1): Xaa is 4-imidazoacetyl (CA)
  MISC_FEATURE (2): Xaa is aminoisobutyric acid (Aib)
  MISC_FEATURE (16)..(20): amino acids at positions 16 and 20 form a ring
XXQGTFTSDYSICMDEKHQKDFVNWLLNTK

SEQ ID NO: 60 - protein, 30 aa, Artificial Sequence
  Trigonal agonist
  MISC_FEATURE (1): Xaa is 4-imidazoacetyl (CA)
  MISC_FEATURE (2): Xaa is aminoisobutyric acid (Aib)
  MISC_FEATURE (16)..(20): amino acids at positions 16 and 20 form a ring
XXQGTFTSDYSIAMDEKHCKDFVNWLLNTK

SEQ ID NO: 61 - protein, 30 aa, Artificial Sequence
  Trigonal agonist
  MISC_FEATURE (1): Xaa is 4-imidazoacetyl (CA)
  MISC_FEATURE (2): Xaa is aminoisobutyric acid (Aib)
  MISC_FEATURE (16)..(20): amino acids at positions 16 and 20 form a ring
XXQGTFTSDYSIAMDEIACKDFVNWLLNTK

SEQ ID NO: 62 - protein, 39 aa, Artificial Sequence
  Trigonal agonist
  MISC_FEATURE (1): Xaa is 4-imidazoacetyl (CA)
  MISC_FEATURE (2): Xaa is aminoisobutyric acid (Aib)
XXQGTFTSDKSKYLDERAAQDFVQWLLDGGPSSGAPPPS

SEQ ID NO: 63 - protein, 39 aa, Artificial Sequence
  Trigonal agonist
  MISC_FEATURE (1): Xaa is 4-imidazoacetyl (CA)
  MISC_FEATURE (2): Xaa is aminoisobutyric acid (Aib)
XXQGTFTSDCSKYLDERAAQDFVQWLLDGGPSSGAPPPS

SEQ ID NO: 64 - protein, 39 aa, Artificial Sequence
  Trigonal agonist
  MISC_FEATURE (2): Xaa is aminoisobutyric acid (Aib)
  MISC_FEATURE (16)..(20): amino acids at positions 16 and 20 form a ring
YXQGTFTSDYSKYLDECAAKEFVQWLLDHHPSSGQPPPS

SEQ ID NO: 65 - protein, 39 aa, Artificial Sequence
  Trigonal agonist
  MISC_FEATURE (2): Xaa is aminoisobutyric acid (Aib)
  MISC_FEATURE (16)..(20): amino acids at positions 16 and 20 form a ring
HXQGTFTSDYSKCLDEKRAKEFVQWLLDHHPSSGQPPPS

SEQ ID NO: 66 - protein, 39 aa, Artificial Sequence
  Trigonal agonist
  MISC_FEATURE (2): Xaa is aminoisobutyric acid (Aib)
  MISC_FEATURE (16)..(20): amino acids at positions 16 and 20 form a ring
YXQGTFTSDYSKYLDECRAKDFVQWLLDHHPSSGQPPPS

SEQ ID NO: 67 - protein, 39 aa, Artificial Sequence
  Trigonal agonist
  MISC_FEATURE (2): Xaa is aminoisobutyric acid (Aib)
  MISC_FEATURE (16)..(20): amino acids at positions 16 and 20 form a ring
YXQGTFTSDYSKYLDECAAKDFVQWLLDHHPSSGQPPPS

SEQ ID NO: 68 - protein, 39 aa, Artificial Sequence
  Trigonal agonist
  MISC_FEATURE (2): Xaa is aminoisobutyric acid (Aib)
  MISC_FEATURE (16)..(20): amino acids at positions 16 and 20 form a ring
YXQGTFTSDYSKCLDEKAAKEFVQWLLDHHPSSGQPPPS

SEQ ID NO: 69 - protein, 39 aa, Artificial Sequence
  Trigonal agonist
  MISC_FEATURE (2): Xaa is aminoisobutyric acid (Aib)
  MISC_FEATURE (16)..(20): amino acids at positions 16 and 20 form a ring
YXQGTFTSDYSKCLDERAAKEFVQWLLDHHPSSGQPPPS

SEQ ID NO: 70 - protein, 39 aa, Artificial Sequence
  Trigonal agonist
  MISC_FEATURE (2): Xaa is aminoisobutyric acid (Aib)
  MISC_FEATURE (16)..(20): amino acids at positions 16 and 20 form a ring
YXQGTFTSDYSKCLDEKRAKDFVQWLLDHHPSSGQPPPS

SEQ ID NO: 71 - protein, 39 aa, Artificial Sequence
  Trigonal agonist
  MISC_FEATURE (2): Xaa is aminoisobutyric acid (Aib)
  MISC_FEATURE (16)..(20): amino acids at positions 16 and 20 form a ring
YXQGTFTSDYSKYLDERACKDFVQWLLDHHPSSGQPPPS

SEQ ID NO: 72 - protein, 39 aa, Artificial Sequence
  Trigonal agonist
  MISC_FEATURE (2): Xaa is aminoisobutyric acid (Aib)
  MISC_FEATURE (16)..(20): amino acids at positions 16 and 20 form a ring
YXQGTFTSDCSKYLDERAAKDFVQWLLDHHPSSGQPPPS

SEQ ID NO: 73 - protein, 39 aa, Artificial Sequence
  Trigonal agonist
  MISC_FEATURE (1): Xaa is 4-imidazoacetyl (CA)
  MISC_FEATURE (2): Xaa is aminoisobutyric acid (Aib)
  MISC_FEATURE (16)..(20): amino acids at positions 16 and 20 form a ring
XXQGTFTSDYSKYLDECRAKEFVQWLLDHHPSSGQPPPS

SEQ ID NO: 74 - protein, 39 aa, Artificial Sequence
  Trigonal agonist
  MISC_FEATURE (1): Xaa is 4-imidazoacetyl (CA)
  MISC_FEATURE (2): Xaa is aminoisobutyric acid (Aib)
  MISC_FEATURE (16)..(20): amino acids at positions 16 and 20 form a ring
XXQGTFTSDYSKCLDEKRAKEFVQWLLDHHPSSGQPPPS

SEQ ID NO: 75 - protein, 40 aa, Artificial Sequence
  Trigonal agonist
  MISC_FEATURE (2): Xaa is aminoisobutyric acid (Aib)
  MISC_FEATURE (16)..(20): amino acids at positions 16 and 20 form a ring
YXQGTFTSDYSKYLDEKAAKEFVQWLLDHHPSSGQPPPSC

SEQ ID NO: 76 - protein, 40 aa, Artificial Sequence
  Trigonal agonist
  MISC_FEATURE (2): Xaa is aminoisobutyric acid (Aib)
  MISC_FEATURE (16)..(20): amino acids at positions 16 and 20 form a ring
YXQGTFTSDYSKYLDEKRAKDFVQWLLDHHPSSGQPPPSC

SEQ ID NO: 77 - protein, 40 aa, Artificial Sequence
  Trigonal agonist
  MISC_FEATURE (2): Xaa is aminoisobutyric acid (Aib)
  MISC_FEATURE (16)..(20): amino acids at positions 16 and 20 form a ring
YXQGTFTSDYSKYLDEKAAKDFVQWLLDHHPSSGQPPPSC

SEQ ID NO: 78 - protein, 31 aa, Artificial Sequence
  Trigonal agonist
  MISC_FEATURE (2): Xaa is aminoisobutyric acid (Aib)
  MISC_FEATURE (16)..(20): amino acids at positions 16 and 20 form a ring
HXQGTFTSDYSKYLDEKRQKEFVQWLLDTKC

SEQ ID NO: 79 - protein, 31 aa, Artificial Sequence
  Trigonal agonist
  MISC_FEATURE (2): Xaa is aminoisobutyric acid (Aib)
  MISC_FEATURE (16)..(20): amino acids at positions 16 and 20 form a ring
HXEGTFTSDYSIAMDEIHQKDFVNWLLAQKC

SEQ ID NO: 80 - protein, 31 aa, Artificial Sequence
  Trigonal agonist
  MISC_FEATURE (2): Xaa is aminoisobutyric acid (Aib)
  MISC_FEATURE (16)..(20): amino acids at positions 16 and 20 form a ring
HXEGTFTSDYSIAMDEIHQKDFVDWLLAEKC

SEQ ID NO: 81 - protein, 30 aa, Artificial Sequence
  Trigonal agonist
  MISC_FEATURE (1): Xaa is 4-imidazoacetyl (CA)
  MISC_FEATURE (2): Xaa is aminoisobutyric acid (Aib)
  MISC_FEATURE (16)..(20): amino acids at positions 16 and 20 form a ring
XXQGTFTSDYSKYLDEKRQKEFVQWLLNTC

SEQ ID NO: 82 - protein, 30 aa, Artificial Sequence
  Trigonal agonist
  MISC_FEATURE (1): Xaa is 4-imidazoacetyl (CA)
  MISC_FEATURE (2): Xaa is aminoisobutyric acid (Aib)
  MISC_FEATURE (16)..(20): amino acids at positions 16 and 20 form a ring
XXQGTFTSDYSKYLDEKRQKEFVQWLLDTC

SEQ ID NO: 83 - protein, 30 aa, Artificial Sequence
  Trigonal agonist
  MISC_FEATURE (1): Xaa is 4-imidazoacetyl (CA)
  MISC_FEATURE (2): Xaa is aminoisobutyric acid (Aib)
  MISC_FEATURE (16)..(20): amino acids at positions 16 and 20 form a ring
XXEGTFTSDYSIAMDEIHQKDFVNWLLAQC

SEQ ID NO: 84 - protein, 30 aa, Artificial Sequence
  Trigonal agonist
  MISC_FEATURE (1): Xaa is 4-imidazoacetyl (CA)
  MISC_FEATURE (2): Xaa is aminoisobutyric acid (Aib)
  MISC_FEATURE (16)..(20): amino acids at positions 16 and 20 form a ring
XXEGTFTSDYSIAMDEIHQKDFVDWLLAEC

SEQ ID NO: 85 - protein, 30 aa, Artificial Sequence
  Trigonal agonist
  MISC_FEATURE (1): Xaa is 4-imidazoacetyl (CA)
  MISC_FEATURE (2): Xaa is aminoisobutyric acid (Aib)
  MISC_FEATURE (16)..(20): amino acids at positions 16 and 20 form a ring
XXQGTFTSDYSIAMDEIHQKDFVNWLLAQC

SEQ ID NO: 86 - protein, 30 aa, Artificial Sequence
  Trigonal agonist
  MISC_FEATURE (1): Xaa is 4-imidazoacetyl (CA)
  MISC_FEATURE (2): Xaa is aminoisobutyric acid (Aib)
  MISC_FEATURE (16)..(20): amino acids at positions 16 and 20 form a ring
XXQGTFTSDYSKYLDEKRQKEFVNWLLAQC

SEQ ID NO: 87 - protein, 30 aa, Artificial Sequence
  Trigonal agonist
  MISC_FEATURE (1): Xaa is 4-imidazoacetyl (CA)
  MISC_FEATURE (2): Xaa is aminoisobutyric acid (Aib)
  MISC_FEATURE (16)..(20): amino acids at positions 16 and 20 form a ring
XXQGTFTSDYSIAMDEIHQKDFVNWLLNTC

SEQ ID NO: 88 - protein, 31 aa, Artificial Sequence
  Trigonal agonist
  MISC_FEATURE (1): Xaa is 4-imidazoacetyl (CA)
  MISC_FEATURE (2): Xaa is aminoisobutyric acid (Aib)
  MISC_FEATURE (16)..(20): amino acids at positions 16 and 20 form a ring
XXQGTFTSDYSKYLDEKRQKEFVQWLLNTKC

SEQ ID NO: 89 - protein, 31 aa, Artificial Sequence
  Trigonal agonist
  MISC_FEATURE (1): Xaa is 4-imidazoacetyl (CA)
  MISC_FEATURE (2): Xaa is aminoisobutyric acid (Aib)
  MISC_FEATURE (16)..(20): amino acids at positions 16 and 20 form a ring
XXQGTFTSDYSKYLDEKRQKEFVQWLLDTKC

SEQ ID NO: 90 - protein, 31 aa, Artificial Sequence
  Trigonal agonist
  MISC_FEATURE (1): Xaa is 4-imidazoacetyl (CA)
  MISC_FEATURE (2): Xaa is aminoisobutyric acid (Aib)
  MISC_FEATURE (16)..(20): amino acids at positions 16 and 20 form a ring
XXEGTFTSDYSIAMDEIHQKDFVNWLLAQKC

SEQ ID NO: 91 - protein, 31 aa, Artificial Sequence
  Trigonal agonist
  MISC_FEATURE (1): Xaa is 4-imidazoacetyl (CA)
  MISC_FEATURE (2): Xaa is aminoisobutyric acid (Aib)
  MISC_FEATURE (16)..(20): amino acids at positions 16 and 20 form a ring
XXEGTFTSDYSIAMDEIHQKDFVDWLLAEKC

SEQ ID NO: 92 - protein, 31 aa, Artificial Sequence
  Trigonal agonist
  MISC_FEATURE (1): Xaa is 4-imidazoacetyl (CA)
  MISC_FEATURE (2): Xaa is aminoisobutyric acid (Aib)
  MISC_FEATURE (16)..(20): amino acids at positions 16 and 20 form a ring
XXQGTFTSDYSIAMDEIHQKDFVNWLLAQKC

SEQ ID NO: 93 - protein, 31 aa, Artificial Sequence
  Trigonal agonist
  MISC_FEATURE (1): Xaa is 4-imidazoacetyl (CA)
  MISC_FEATURE (2): Xaa is aminoisobutyric acid (Aib)
  MISC_FEATURE (16)..(20): amino acids at positions 16 and 20 form a ring
XXQGTFTSDYSKYLDEKRQKEFVNWLLAQKC

SEQ ID NO: 94 - protein, 31 aa, Artificial Sequence
  Trigonal agonist
  MISC_FEATURE (1): Xaa is 4-imidazoacetyl (CA)
  MISC_FEATURE (2): Xaa is aminoisobutyric acid (Aib)
  MISC_FEATURE (16)..(20): amino acids at positions 16 and 20 form a ring
XXQGTFTSDYSIAMDEIHQKDFVNWLLNTKC

SEQ ID NO: 95 - protein, 39 aa, Artificial Sequence
  Trigonal agonist
  MISC_FEATURE (2): Xaa is aminoisobutyric acid (Aib)
  MISC_FEATURE (16)..(20): amino acids at positions 16 and 20 form a ring
YXQGTFTSDYSKYLDEKRAKEFVQWLLCHHPSSGQPPPS

SEQ ID NO: 96 - protein, 39 aa, Artificial Sequence
  Trigonal agonist
  MISC_FEATURE (2): Xaa is aminoisobutyric acid (Aib)
  MISC_FEATURE (16)..(20): amino acids at positions 16 and 20 form a ring
YXQGTFTSDYSKYLDEKRAKEFVQWLLDHCPSSGQPPPS

SEQ ID NO: 97 - protein, 39 aa, Artificial Sequence
  Trigonal agonist
  MISC_FEATURE (2): Xaa is aminoisobutyric acid (Aib)
  MISC_FEATURE (16)..(20): amino acids at positions 16 and 20 form a ring
YXQGTFTSDYSKYLDEKRAKEFVQWLLDCHPSSGQPPPS

SEQ ID NO: 98 - protein, 40 aa, Artificial Sequence
  Trigonal agonist
  MISC_FEATURE (2): Xaa is aminoisobutyric acid (Aib)
  MISC_FEATURE (16)..(20): amino acids at positions 16 and 20 form a ring
YXQGTFTSDYSKALDEKAAKEFVNWLLDHHPSSGQPPPSC

SEQ ID NO: 99 - protein, 40 aa, Artificial Sequence
  Trigonal agonist
  MISC_FEATURE (2): Xaa is aminoisobutyric acid (Aib)
  MISC_FEATURE (16)..(20): amino acids at positions 16 and 20 form a ring
YXQGTFTSDYSKALDEKAAKDFVNWLLDHHPSSGQPPPSC

SEQ ID NO: 100 - protein, 40 aa, Artificial Sequence
  Trigonal agonist
  MISC_FEATURE (2): Xaa is aminoisobutyric acid (Aib)
  MISC_FEATURE (16)..(20): amino acids at positions 16 and 20 form a ring
YXQGTFTSDYSKALDEKAAKEFVQWLLDQHPSSGQPPPSC

SEQ ID NO: 101 - protein, 40 aa, Artificial Sequence
  Trigonal agonist
  MISC_FEATURE (2): Xaa is aminoisobutyric acid (Aib)
  MISC_FEATURE (16)..(20): amino acids at positions 16 and 20 form a ring
YXQGTFTSDYSKALDEKAAKEFVNWLLDQHPSSGQPPPSC

SEQ ID NO: 102 - protein, 40 aa, Artificial Sequence
  Trigonal agonist
  MISC_FEATURE (2): Xaa is aminoisobutyric acid (Aib)
  MISC_FEATURE (16)..(20): amino acids at positions 16 and 20 form a ring
YXQGTFTSDYSKALDEKAAKDFVNWLLDQHPSSGQPPPSC

SEQ ID NO: 103 - protein, 30 aa, Artificial Sequence
  General Formula 1
  MISC_FEATURE (1): Xaa is His (H), 4-imidazoacetyl (CA), or Tyr (Y)
  MISC_FEATURE (2): Xaa is Gly (G), alpha-methyl-glutamic acid, or Aib (aminoisobutyric acid)
  MISC_FEATURE (3): Xaa is Glu (E) or Gln (Q)
  MISC_FEATURE (7): Xaa is Thr (T) or Ile (I)
  MISC_FEATURE (10): Xaa is Leu (L), Tyr (Y), Lys (K), Cys (C), or Val (V)
  MISC_FEATURE (12): Xaa is Lys (K), Ser (S), or Ile (I)
  MISC_FEATURE (13): Xaa is Gln (Q), Tyr (Y), Ala (A), or Cys (C)
  MISC_FEATURE (14): Xaa is Leu (L), Met (M), or Tyr (Y)
  MISC_FEATURE (15): Xaa is Cys (C), Asp (D), Glu (E), or Leu (L)
  MISC_FEATURE (16): Xaa is Gly (G), Glu (E), or Ser (S)
  MISC_FEATURE (17): Xaa is Gln (Q), Arg (R), Ile (I), Glu (E), Cys (C), or Lys (K)
  MISC_FEATURE (18): Xaa is Ala (A), Gln (Q), Arg (R), or His (H)
  MISC_FEATURE (19): Xaa is Ala (A), Gln (Q), Cys (C), or Val (V)
  MISC_FEATURE (20): Xaa is Lys (K), Gln (Q), or Arg (R)
  MISC_FEATURE (21): Xaa is Glu (E), Gln (Q), Leu (L), Cys (C), or Asp (D)
  MISC_FEATURE (23): Xaa is Ile (I) or Val (V)
  MISC_FEATURE (24): Xaa is Ala (A), Gln (Q), Cys (C), Asn (N), Asp (D), or Glu (E)
  MISC_FEATURE (27): Xaa is Val (V), Leu (L), Lys (K), or Met (M)
  MISC_FEATURE (28): Xaa is Cys (C), Lys (K), Ala (A), Asn (N), or Asp (D)
  MISC_FEATURE (29): Xaa is Cys (C), Gly (G), Gln (Q), Thr (T), Glu (E), or His (H)
  MISC_FEATURE (30): Xaa is Cys (C), Gly (G), Lys (K), or His (H), or is absent; and Xaa can be further linked to R1, wherein R1 is Cys (C), GKKNDWKHNIT, m-SSGAPPPS-n, or m-SSGQPPPS-n, or is absent, and wherein m is -Cys-, -Pro-, or -Gly-Pro-, and n is -Cys-, -Gly-, -Ser-, or -His
XXXGTFXSDXSXXXXXXXXXXFXXWLXXXX

SEQ ID NO: 104 - protein, 40 aa, Artificial Sequence
  General Formula 2
  MISC_FEATURE (1): Xaa is His (H), 4-imidazoacetyl (CA), or Tyr (Y)
  MISC_FEATURE (2): Xaa is Gly (G), alpha-methyl-glutamic acid, or Aib (aminoisobutyric acid)
  MISC_FEATURE (10): Xaa is Tyr (Y) or Cys (C)
  MISC_FEATURE (13): Xaa is Gln (Q), Tyr (Y), Ala (A), or Cys (C)
  MISC_FEATURE (14): Xaa is Leu (L), Met (M), or Tyr (Y)
  MISC_FEATURE (15): Xaa is Asp (D), Glu (E), or Leu (L)
  MISC_FEATURE (16): Xaa is Gly (G), Glu (E), or Ser (S)
  MISC_FEATURE (17): Xaa is Gln (Q), Arg (R), Ile (I), Glu (E), Cys (C), or Lys (K)
  MISC_FEATURE (18): Xaa is Ala (A), Gln (Q), Arg (R), or His (H)
  MISC_FEATURE (19): Xaa is Ala (A), Gln (Q), Cys (C), or Val (V)
  MISC_FEATURE (20): Xaa is Lys (K), Gln (Q), or Arg (R)
  MISC_FEATURE (21): Xaa is Glu (E), Gln (Q), Leu (L), Cys (C), or Asp (D)
  MISC_FEATURE (23): Xaa is Ile (I) or Val (V)
  MISC_FEATURE (24): Xaa is Ala (A), Gln (Q), Cys (C), Asn (N), or Glu (E)
  MISC_FEATURE (28): Xaa is Cys (C), Lys (K), Asn (N), or Asp (D)
  MISC_FEATURE (29): Xaa is Cys (C), Gly (G), Gln (Q), or His (H)
  MISC_FEATURE (30): Xaa is Cys (C), Gly (G), Lys (K), or His (H)
  MISC_FEATURE (31): Xaa is Pro (P) or Cys (C)
  MISC_FEATURE (40): Xaa is Cys (C), or is absent
XXQGTFTSDXSKXXXXXXXXXFXXWLLXXXXSSGQPPPSX

SEQ ID NO: 105 - protein, 40 aa, Artificial Sequence
  General Formula 3
  MISC_FEATURE (1): Xaa is His (H) or Tyr (Y)
  MISC_FEATURE (2): Xaa is alpha-methyl-glutamic acid, or Aib (aminoisobutyric acid)
  MISC_FEATURE (13): Xaa is Tyr (Y), Ala (A), or Cys (C)
  MISC_FEATURE (17): Xaa is Arg (R), Cys (C), or Lys (K)
  MISC_FEATURE (18): Xaa is Ala (A) or Arg (R)
  MISC_FEATURE (19): Xaa is Ala (A) or Cys (C)
  MISC_FEATURE (21): Xaa is Glu (E) or Asp (D)
  MISC_FEATURE (24): Xaa is Gln (Q) or Asn (N)
  MISC_FEATURE (28): Xaa is Cys (C) or Asp (D)
  MISC_FEATURE (29): Xaa is Cys (C), Gln (Q), or His (H)
  MISC_FEATURE (30): Xaa is Cys (C) or His (H)
  MISC_FEATURE (31): Xaa is Pro (P) or Cys (C)
  MISC_FEATURE (40): Xaa is Cys (C), or is absent
XXQGTFTSDYSKXLDEXXXKXFVXWLLXXXXSSGQPPPSX

SEQ ID NO: 106 - protein, 11 aa, Artificial Sequence
  R1
GKKNDWKHNIT

SEQ ID NO: 107 - protein, 8 aa, Artificial Sequence
  R1
SSGAPPPS

SEQ ID NO: 108 - protein, 8 aa, Artificial Sequence
  R1
SSGQPPPS

SEQ ID NO: 109 - protein, 9 aa, Artificial Sequence
  R1
CSSGQPPPS

SEQ ID NO: 110 - protein, 10 aa, Artificial Sequence
  R1
GPSSGAPPPS

SEQ ID NO: 111 - protein, 11 aa, Artificial Sequence
  R1
GPSSGAPPPSC

SEQ ID NO: 112 - protein, 9 aa, Artificial Sequence
  R1
PSSGAPPPS

SEQ ID NO: 113 - protein, 10 aa, Artificial Sequence
  R1
PSSGAPPPSG

SEQ ID NO: 114 - protein, 11 aa, Artificial Sequence
  R1
PSSGAPPPSHG

SEQ ID NO: 115 - protein, 10 aa, Artificial Sequence
  R1
PSSGAPPPSS

SEQ ID NO: 116 - protein, 9 aa, Artificial Sequence
  R1
PSSGQPPPS

SEQ ID NO: 117 - protein, 10 aa, Artificial Sequence
  R1
PSSGQPPPSC

SEQ ID NO: 118 - protein, 29 aa, Homo sapiens
HSQGTFTSDYSKYLDSRRAQDFVQWLMNT

SEQ ID NO: 119 - protein, 12 aa, HOMO SAPIENS
ESKYGPPCPSCP

SEQ ID NO: 120 - protein, 11 aa, Artificial Sequence
  Variant of hinge region
ESKYGPPPSCP

SEQ ID NO: 121 - protein, 11 aa, Artificial Sequence
  Variant of hinge region
ESKYGPPCPSP

SEQ ID NO: 122 - protein, 10 aa, Artificial Sequence
  Variant of hinge region
ESKYGPPCPS

SEQ ID NO: 123 - protein, 10 aa, Artificial Sequence
  Variant of hinge region
ESKYGPPCPP

SEQ ID NO: 124 - protein, 8 aa, Artificial Sequence
  Variant of hinge region
KYGPPCPS

SEQ ID NO: 125 - protein, 8 aa, Artificial Sequence
  Variant of hinge region
ESKYGPPC

SEQ ID NO: 126 - protein, 7 aa, Artificial Sequence
  Variant of hinge region
EKYGPPC

SEQ ID NO: 127 - protein, 6 aa, Artificial Sequence
  Variant of hinge region
ESPSCP

SEQ ID NO: 128 - protein, 5 aa, Artificial Sequence
  Variant of hinge region
EPSCP

SEQ ID NO: 129 - protein, 4 aa, Artificial Sequence
  Variant of hinge region
PSCP

SEQ ID NO: 130 - protein, 10 aa, Artificial Sequence
  Variant of hinge region
ESKYGPPSCP

SEQ ID NO: 131 - protein, 9 aa, Artificial Sequence
  Variant of hinge region
KYGPPPSCP

SEQ ID NO: 132 - protein, 9 aa, Artificial Sequence
  Variant of hinge region
ESKYGPSCP

SEQ ID NO: 133 - protein, 8 aa, Artificial Sequence
  Variant of hinge region
ESKYGPPC

SEQ ID NO: 134 - protein, 7 aa, Artificial Sequence
  Variant of hinge region
KYGPPCP

SEQ ID NO: 135 - protein, 7 aa, Artificial Sequence
  Variant of hinge region
ESKPSCP

SEQ ID NO: 136 - protein, 6 aa, Artificial Sequence
  Variant of hinge region
ESPSCP

SEQ ID NO: 137 - protein, 4 aa, Artificial Sequence
  Variant of hinge region
EPSC

SEQ ID NO: 138 - protein, 3 aa, Artificial Sequence
  Variant of hinge region
SCP

SEQ ID NO: 139 - protein, 221 aa, homo sapiens
PSCPAPEFLGGPSVFLFPPKPKDTLMISRTPEVTCVVVDVSQEDPEVQFNWYVDGVEVHNAKTKPREEQFNSTYRVVSVLTVLHQDWLNGKEYKCKVSNKGLPSSIEKTISKAKGQPREPQVYTLPPSQEEMTKNQVSLTCLVKGFYPSDIAVEWESNGQPENNYKTTPPVLDSDGSFFLYSRLTVDKSRWQEGNVFSCSVMHEALHNHYTQKSLSLSLGK